European Patent Specification EP 3 125 943 B1, published April 22, 2026. Title: PHOSPHATE BASED LINKERS FOR INTRACELLULAR DELIVERY OF DRUG CONJUGATES. Applicant: Merck Sharp & Dohme Corp. Ambrx, Inc. Garbaccio, Robert M Kern, Jeffrey Brandish, Philip E Shah, Sanjiv Liang, Linda Sun, Ying Wang, Jianing Knudsen, Nick Beck, Andrew Manibusan, Anthony Gately, Dennis. The sequence listing filed with the application follows.

SEQUENCE LISTING (4 sequences)

SEQ ID NO: 1 - protein, 447 aa, artificial sequence
  Anti-CD70 2H5 IgG1
  MOD_RES (119)..(119): Xaa is para-azido-phenylalanine (pAF)
QVQLVESGGGVVQPGRSLRLSCAASGFTFSSYIMHWVRQAPGKGLEWVAVISYDGRNKYYADSVKGRFTISRDNSKNTLYLQMNSLRAEDTAVYYCARDTDGYDFDYWGQGTLVTVSSXSTKGPSVFPLAPSSKSTSGGTAALGCLVKDYFPEPVTVSWNSGALTSGVHTFPAVLQSSGLYSLSSVVTVPSSSLGTQTYICNVNHKPSNTKVDKKVEPKSCDKTHTCPPCPAPELLGGPSVFLFPPKPKDTLMISRTPEVTCVVVDVSHEDPEVKFNWYVDGVEVHNAKTKPREEQYNSTYRVVSVLTVLHQDWLNGKEYKCKVSNKALPAPIEKTISKAKGQPREPQVYTLPPSRDELTKNQVSLTCLVKGFYPSDIAVEWESNGQPENNYKTTPPVLDSDGSFFLYSKLTVDKSRWQQGNVFSCSVMHEALHNHYTQKSLSLSPG

SEQ ID NO: 2 - protein, 214 aa, Artificial Sequence
  Anti-CD70 Kappa Light chain
EIVLTQSPATLSLSPGERATLSCRASQSVSSYLAWYQQKPGQAPRLLIYDASNRATGIPARFSGSGSGTDFTLTISSLEPEDFAVYYCQQRTNWPLTFGGGTKVEIKRTVAAPSVFIFPPSDEQLKSGTASVVCLLNNFYPREAKVQWKVDNALQSGNSQESVTEQDSKDSTYSLSSTLTLSKADYEKHKVYACEVTHQGLSSPVTKSFNRGEC

SEQ ID NO: 3 - protein, 438 aa, artificial Sequence
  Anti-murine CD25 muIgG1 D265A
  MOD_RES (115)..(115): Xaa is para-azido-phenylalanine (pAF)
QVKLLQSGAALVKPGASVKMSCKASGYSFPDSWVTWVKQSHGKSLEWIGDIFPNSGATNFNEKFKGKATLTVDKSTSTAYMELSRLTSEDSAIYYCTRLDYGYWGQGVMVTVSSXKTTPPSVYPLAPGSAAQTNSMVTLGCLVKGYFPEPVTVTWNSGSLSSGVHTFPAVLQSDLYTLSSSVTVPSSTWPSETVTCNVAHPASSTKVDKKIVPRDCGCKPCICTVPEVSSVFIFPPKPKDVLTITLTPKVTCVVVAISKDDPEVQFSWFVDDVEVHTAQTQPREEQFNSTFRSVSELPIMHQDWLNGKEFKCRVNSAAFPAPIEKTISKTKGRPKAPQVYTIPPPKEQMAKDKVSLTCMITDFFPEDITVEWQWNGQPAENYKNTQPIMDTDGSYFVYSKLNVQKSNWEAGNTFTCSVLHEGLHNHHTEKSLSHSPGK

SEQ ID NO: 4 - protein, 219 aa, Artificial Sequence
  Anti-murine CD25 muKappa
DVVLTQTPPTLSATIGQSVSISCRSSQSLLHSNGNTYLNWLLQRPGQPPQLLIYLASRLESGVPNRFSGSGSGTDFTLKISGVEAEDLGVYYCVQSSHFPNTFGVGTKLELKRADAAPTVSIFPPSSEQLTSGGASVVCFLNNFYPKDINVKWKIDGSERQNGVLNSWTDQDSKDSTYSMSSTLTLTKDEYERHNSYTCEATHKTSTSPIVKSFNRNEC